European Patent Specification EP 4 370 593 B1, published September 10, 2025. Title: Method to degrade plastic. Applicant: Repsol S.A. The sequence listing filed with the application follows.

SEQUENCE LISTING (4 sequences)

SEQ ID NO: 1 - protein, 236 aa, Marasmius rotula
SAHPWKAPGPNDSRGPCPGLNTLANHGFLPRNGRNISVPMIVKAGFEGYNVQSDILILAGKIGMLTSREADTISLEDLKLHGTIEHDASLSREDVAIGDNLHFNEAIFTTLANSNPGADVYNISSAAQVQHDRLADSLARNPNVTNTDLTATIRSSESAFFLTVMSAGDPLRGEAPKKFVNVFFREERMPIKEGWKRSTTPITIPLLGPIIERITELSDWKPTGDNCGAIVLSPEL

SEQ ID NO: 2 - protein, 328 aa, Agrocybe aegerita
EPGLPPGPLENSSAKLVNDEAHPWKPLRPGDIRGPCPGLNTLASHGYLPRNGVATPAQIINAVQEGFNFDNQAAIFATYAAHLVDGNLITDLLSIGRKTRLTGPDPPPPASVGGLNEHGTFEGDASMTRGDAFFGNNHDFNETLFEQLVDYSNRFGGGKYNLTVAGELRFKRIQDSIATNPNFSFVDFRFFTAYGETTFPANLFVDGRRDDGQLDMDAARSFFQFSRMPDDFFRAPSPRSGTGVEVVVQAHPMQPGRNVGKINSYTVDPTSSDFSTPCLMYEKFVNITVKSLYPNPTVQLRKALNTNLDFLFQGVAAGCTQVFPYGRD

SEQ ID NO: 3 - protein, 496 aa, synthetic construct
  REGION 1..496: note = evolved laccase
SIGPVADLTISNGAVSPDGFSRQAILVNDVFPSPLITGNKGDRFQLNVIDNMTNHTMLKSTSIHWHGFFQHGTNWADGPAFVNQCPISTGHAFLYDFQVPDQAGTFWYHSHLSTQYCDGLRGPIVVYDPQDPHKSLYDVDDDSTVITLADWYHLAAKVGPAAPTADATLINGLGRSINTLNADLAVITVTKGKRYRFRLVSLSCDPNYTFSIDGHSLTVIEADGVNLKPQTVDSIQIFPAQRYSFVLNADQDVDNYWIRALPNSGTRNFDGGVNSAILRYEGAAPVEPTTTQTPSTQPLVESALTTLEGTAAPGNPTPGGVDLALNMAFGFAGGRFTINGASFTPPTVPVLLQILSGAQSAQDLLPSGSVYSLPANADIEISLPATSAAPGFPHPFHLHGHTFAVVRSAGSSTYNYANPVYRDVVNTGSPGDNVTIRFRTDNPGPWFLHCHIDFHLEAGFTVVMAEDIPDVAATNPVPQAWSDLCPTYDALSPDDQ

SEQ ID NO: 4 - protein, 403 aa, synthetic construct
  REGION 1..403: note = evolved versatile peroxidase
APVNTTTEDETAQIPAEAVIGYSDLEGDFDVAVLPFSNSTNNGLLFINTTIASIAAKEEGVSLEKREAEAEFATCDDGRTTANAACCILFPILDDIQENLFDGAQCGEKVHESLRLTFHDAIGFSPTLGGGGADGSIIAFDTIETNFPANAGIDEIVSAQKPFVAKHNISAGDFIQFAGAVGVSNCPGGVRIPFFLGRPDAVAASPDHLVPEPFDSVDSILARMGDAGFSPAEVVWLLASHSIAAADKVDPSIPGMPFDSTPGVFDSQFFIETLLKGRLFPGTADNKGEAQSPLQGEIRLQSDHLLARDPQTACEWQSMVNNQPKIQNRFAATMSKMALLGQDKTKLIDCSDVIPTPPALVGAAHLPAGFSLSDVEQACAATPFPALTADPGPVTSVPPVPGS